European Patent Application EP 4 650 451 A1, published November 19, 2025. Title: MRNA MOLECULE FOR TARGETED PROTEIN DEGRADATION, AND USE. Applicant: COSYCHEM BIOTECHNOLOGY TECHNOLOGY (TIANJIN) CO., LTD. Application WO PCT/CN2024/070318, filed January 3, 2024. The sequence listing filed with the application follows.

SEQUENCE LISTING (15 sequences)

SEQ ID NO: 1 - protein, 7 aa, Artificial sequence
PIYPALA

SEQ ID NO: 2 - protein, 4 aa, Artificial sequence
GSGS

SEQ ID NO: 3 - protein, 6 aa, Artificial sequence
GGGGGG

SEQ ID NO: 4 - protein, 9 aa, Artificial sequence
QLLRHLILH

SEQ ID NO: 5 - protein, 16 aa, Artificial sequence
GQVGRQLAIIGDAINR

SEQ ID NO: 6 - protein, 20 aa, Artificial sequence
PIYPALAGSGSQLLRHLILH

SEQ ID NO: 7 - RNA, 1037 nt, Artificial sequence
  source 1..1037: mol_type = mRNA
acatttgcttctgacacaactgtgttcactagcaacctcaaagagacaccgccaccatggtgagcaagggcgaggagctgttcaccggggtggtgcccatcctggtcgagctggacggcgacgtaaacggccacaagttcagcgtgtccggcgagggcgagggcgatgccacctacggcaagctgaccctgaagttcatctgcaccaccggcaagctgcccgtgccctggcccaccctcgtgaccaccctgacctacggcgtgcagtgcttcagccgctaccccgaccacatgaagcagcacgacttcttcaagtccgccatgcccgaaggctacgtccaggagcgcaccatcttcttcaaggacgacggcaactacaagacccgcgccgaggtgaagttcgagggcgacaccctggtgaaccgcatcgagctgaagggcatcgacttcaaggaggacggcaacatcctggggcacaagctggagtacaactacaacagccacaacgtctatatcatggccgacaagcagaagaacggcatcaaggtgaacttcaagatccgccacaacatcgaggacggcagcgtgcagctcgccgaccactaccagcagaacacccccatcggcgacggccccgtgctgctgcccgacaaccactacctgagcacccagtccgccctgagcaaagaccccaacgagaagcgcgatcacatggtcctgctggagttcgtgaccgccgccgggatcactctcggcatggacgagctgtacaagggaagcggagccacgaacttctctctgttaaagcaagcaggagatgttgaagaaaaccccgggcctatctaccccgccctggccggctccggctcccagctgctgcgccacctgatcctgcactgagctggagcctcggtagccgttcctcctgcccgctgggcctcccaacgggccctcctcccctccttgcaccggcccttcctggtctttgaataaagtctgagtgggcggaaaaaaaaaaaaaaaaaaaaaaaaaaaaaa

SEQ ID NO: 8 - DNA, 1037 bp, Artificial sequence
  source 1..1037: mol_type = other DNA
acatttgcttctgacacaactgtgttcactagcaacctcaaagagacaccgccaccatggtgagcaagggcgaggagctgttcaccggggtggtgcccatcctggtcgagctggacggcgacgtaaacggccacaagttcagcgtgtccggcgagggcgagggcgatgccacctacggcaagctgaccctgaagttcatctgcaccaccggcaagctgcccgtgccctggcccaccctcgtgaccaccctgacctacggcgtgcagtgcttcagccgctaccccgaccacatgaagcagcacgacttcttcaagtccgccatgcccgaaggctacgtccaggagcgcaccatcttcttcaaggacgacggcaactacaagacccgcgccgaggtgaagttcgagggcgacaccctggtgaaccgcatcgagctgaagggcatcgacttcaaggaggacggcaacatcctggggcacaagctggagtacaactacaacagccacaacgtctatatcatggccgacaagcagaagaacggcatcaaggtgaacttcaagatccgccacaacatcgaggacggcagcgtgcagctcgccgaccactaccagcagaacacccccatcggcgacggccccgtgctgctgcccgacaaccactacctgagcacccagtccgccctgagcaaagaccccaacgagaagcgcgatcacatggtcctgctggagttcgtgaccgccgccgggatcactctcggcatggacgagctgtacaagggaagcggagccacgaacttctctctgttaaagcaagcaggagatgttgaagaaaaccccgggcctatctaccccgccctggccggctccggctcccagctgctgcgccacctgatcctgcactgagctggagcctcggtagccgttcctcctgcccgctgggcctcccaacgggccctcctcccctccttgcaccggcccttcctggtctttgaataaagtctgagtgggcggaaaaaaaaaaaaaaaaaaaaaaaaaaaaaa

SEQ ID NO: 9 - DNA, 3087 bp, Artificial sequence
  source 1..3087: mol_type = other DNA
taatacgactcactataggacatttgcttctgacacaactgtgttcactagcaacctcaaagagacaccgccaccatggtgagcaagggcgaggagctgttcaccggggtggtgcccatcctggtcgagctggacggcgacgtaaacggccacaagttcagcgtgtccggcgagggcgagggcgatgccacctacggcaagctgaccctgaagttcatctgcaccaccggcaagctgcccgtgccctggcccaccctcgtgaccaccctgacctacggcgtgcagtgcttcagccgctaccccgaccacatgaagcagcacgacttcttcaagtccgccatgcccgaaggctacgtccaggagcgcaccatcttcttcaaggacgacggcaactacaagacccgcgccgaggtgaagttcgagggcgacaccctggtgaaccgcatcgagctgaagggcatcgacttcaaggaggacggcaacatcctggggcacaagctggagtacaactacaacagccacaacgtctatatcatggccgacaagcagaagaacggcatcaaggtgaacttcaagatccgccacaacatcgaggacggcagcgtgcagctcgccgaccactaccagcagaacacccccatcggcgacggccccgtgctgctgcccgacaaccactacctgagcacccagtccgccctgagcaaagaccccaacgagaagcgcgatcacatggtcctgctggagttcgtgaccgccgccgggatcactctcggcatggacgagctgtacaagggaagcggagccacgaacttctctctgttaaagcaagcaggagatgttgaagaaaaccccgggcctatctaccccgccctggccggctccggctcccagctgctgcgccacctgatcctgcactgagctggagcctcggtagccgttcctcctgcccgctgggcctcccaacgggccctcctcccctccttgcaccggcccttcctggtctttgaataaagtctgagtgggcggaaaaaaaaaaaaaaaaaaaaaaaaaaaaaatgaagagccgtacgggcgcgcctaggcgcgattccgcttcctcgctcactgactcgctgcgctcggtcgttcggctgcggcgagcggtatcagctcactcaaaggcggtaatacggttatccacagaatcaggggataacgcaggaaagaacatgtgagcaaaaggccagcaaaaggccaggaaccgtaaaaaggccgcgttgctggcgtttttccataggctccgcccccctgacgagcatcacaaaaatcgacgctcaagtcagaggtggcgaaacccgacaggactataaagataccaggcgtttccccctggaagctccctcgtgcgctctcctgttccgaccctgccgcttaccggatacctgtccgcctttctcccttcgggaagcgtggcgctttctcatagctcacgctgtaggtatctcagttcggtgtaggtcgttcgctccaagctgggctgtgtgcacgaaccccccgttcagcccgaccgctgcgccttatccggtaactatcgtcttgagtccaacccggtaagacacgacttatcgccactggcagcagccactggtaacaggattagcagagcgaggtatgtaggcggtgctacagagttcttgaagtggtggcctaactacggctacactagaagaacagtatttggtatctgcgctctgctgaagccagttaccttcggaaaaagagttggtagctcttgatccggcaaacaaaccaccgctggtagcggtggtttttttgtttgcaagcagcagattacgcgcagaaaaaaaggatctcaagaagatcctttgatcttttctacggggtctgacgctcagtggaacgaaaactcacgttaagggattttggtcatgagattatcaaaaaggatcttcacctagatccttttaaattaaaaatgaagttttaaatcaatctaaagtatatatgagtaaacttggtctgacagttaccaatgcttaatcagtgaggcacctatctcagcgatctgtctatttcgttcatccatagttgcctgactccccgtcgtgtagataactacgatacgggagggcttaccatctggccccagtgctgcaatgataccgcgagatccacgctcaccggctccagatttatcagcaataaaccagccagccggaagggccgagcgcagaagtggtcctgcaactttatccgcctccatccagtctattaattgttgccgggaagctagagtaagtagttcgccagttaatagtttgcgcaacgttgttgccattgctacaggcatcgtggtgtcacgctcgtcgtttggtatggcttcattcagctccggttcccaacgatcaaggcgagttacatgatcccccatgttgtgcaaaaaagcggttagctccttcggtcctccgatcgttgtcagaagtaagttggccgcagtgttatcactcatggttatggcagcactgcataattctcttactgtcatgccatccgtaagatgcttttctgtgactggtgagtactcaaccaagtcattctgagaatagtgtatgcggcgaccgagttgctcttgcccggcgtcaatacgggataataccgcgccacatagcagaactttaaaagtgctcatcattggaaaacgttcttcggggcgaaaactctcaaggatcttaccgctgttgagatccagttcgatgtaacccactcgtgcacccaactgatcttcagcatcttttactttcaccagcgtttctgggtgagcaaaaacaggaaggcaaaatgccgcaaaaaagggaataagggcgacacggaaatgttgaatactcatactcttcctttttcaatattattgaagcatttatcagggttattgtctcatgagcggatacatatttgaatgtatttagaaaaataaacaaataggggttccgcgcacatttccccgaaaagtgccacctgacgtctaagaaaccattattatcatgacattaacctataaaaataggcgtatcacgaggccctttcgtc

SEQ ID NO: 10 - DNA, 980 bp, Artificial sequence
  source 1..980: mol_type = other DNA
acatttgcttctgacacaactgtgttcactagcaacctcaaagagacaccgccaccatggtgagcaagggcgaggagctgttcaccggggtggtgcccatcctggtcgagctggacggcgacgtaaacggccacaagttcagcgtgtccggcgagggcgagggcgatgccacctacggcaagctgaccctgaagttcatctgcaccaccggcaagctgcccgtgccctggcccaccctcgtgaccaccctgacctacggcgtgcagtgcttcagccgctaccccgaccacatgaagcagcacgacttcttcaagtccgccatgcccgaaggctacgtccaggagcgcaccatcttcttcaaggacgacggcaactacaagacccgcgccgaggtgaagttcgagggcgacaccctggtgaaccgcatcgagctgaagggcatcgacttcaaggaggacggcaacatcctggggcacaagctggagtacaactacaacagccacaacgtctatatcatggccgacaagcagaagaacggcatcaaggtgaacttcaagatccgccacaacatcgaggacggcagcgtgcagctcgccgaccactaccagcagaacacccccatcggcgacggccccgtgctgctgcccgacaaccactacctgagcacccagtccgccctgagcaaagaccccaacgagaagcgcgatcacatggtcctgctggagttcgtgaccgccgccgggatcactctcggcatggacgagctgtacaagggaagcggagccacgaacttctctctgttaaagcaagcaggagatgttgaagaaaaccccgggccttgagctggagcctcggtagccgttcctcctgcccgctgggcctcccaacgggccctcctcccctccttgcaccggcccttcctggtctttgaataaagtctgagtgggcggaaaaaaaaaaaaaaaaaaaaaaaaaaaaaa

SEQ ID NO: 11 - protein, 29 aa, Artificial sequence
PIYPALAGGGGGGGQVGRQLAIIGDAINR

SEQ ID NO: 12 - RNA, 1064 nt, Artificial sequence
  source 1..1064: mol_type = mRNA
acatttgcttctgacacaactgtgttcactagcaacctcaaagagacaccgccaccatggtgagcaagggcgaggagctgttcaccggggtggtgcccatcctggtcgagctggacggcgacgtaaacggccacaagttcagcgtgtccggcgagggcgagggcgatgccacctacggcaagctgaccctgaagttcatctgcaccaccggcaagctgcccgtgccctggcccaccctcgtgaccaccctgacctacggcgtgcagtgcttcagccgctaccccgaccacatgaagcagcacgacttcttcaagtccgccatgcccgaaggctacgtccaggagcgcaccatcttcttcaaggacgacggcaactacaagacccgcgccgaggtgaagttcgagggcgacaccctggtgaaccgcatcgagctgaagggcatcgacttcaaggaggacggcaacatcctggggcacaagctggagtacaactacaacagccacaacgtctatatcatggccgacaagcagaagaacggcatcaaggtgaacttcaagatccgccacaacatcgaggacggcagcgtgcagctcgccgaccactaccagcagaacacccccatcggcgacggccccgtgctgctgcccgacaaccactacctgagcacccagtccgccctgagcaaagaccccaacgagaagcgcgatcacatggtcctgctggagttcgtgaccgccgccgggatcactctcggcatggacgagctgtacaagggaagcggagccacgaacttctctctgttaaagcaagcaggagatgttgaagaaaaccccgggcctatttatcctgctctggccgggggcggaggaggcggcggccaggtgggaagacagctggccattattggggatgccattaatagatgagctggagcctcggtagccgttcctcctgcccgctgggcctcccaacgggccctcctcccctccttgcaccggcccttcctggtctttgaataaagtctgagtgggcggaaaaaaaaaaaaaaaaaaaaaaaaaaaaaa

SEQ ID NO: 13 - DNA, 1064 bp, Artificial sequence
  source 1..1064: mol_type = other DNA
acatttgcttctgacacaactgtgttcactagcaacctcaaagagacaccgccaccatggtgagcaagggcgaggagctgttcaccggggtggtgcccatcctggtcgagctggacggcgacgtaaacggccacaagttcagcgtgtccggcgagggcgagggcgatgccacctacggcaagctgaccctgaagttcatctgcaccaccggcaagctgcccgtgccctggcccaccctcgtgaccaccctgacctacggcgtgcagtgcttcagccgctaccccgaccacatgaagcagcacgacttcttcaagtccgccatgcccgaaggctacgtccaggagcgcaccatcttcttcaaggacgacggcaactacaagacccgcgccgaggtgaagttcgagggcgacaccctggtgaaccgcatcgagctgaagggcatcgacttcaaggaggacggcaacatcctggggcacaagctggagtacaactacaacagccacaacgtctatatcatggccgacaagcagaagaacggcatcaaggtgaacttcaagatccgccacaacatcgaggacggcagcgtgcagctcgccgaccactaccagcagaacacccccatcggcgacggccccgtgctgctgcccgacaaccactacctgagcacccagtccgccctgagcaaagaccccaacgagaagcgcgatcacatggtcctgctggagttcgtgaccgccgccgggatcactctcggcatggacgagctgtacaagggaagcggagccacgaacttctctctgttaaagcaagcaggagatgttgaagaaaaccccgggcctatttatcctgctctggccgggggcggaggaggcggcggccaggtgggaagacagctggccattattggggatgccattaatagatgagctggagcctcggtagccgttcctcctgcccgctgggcctcccaacgggccctcctcccctccttgcaccggcccttcctggtctttgaataaagtctgagtgggcggaaaaaaaaaaaaaaaaaaaaaaaaaaaaaa

SEQ ID NO: 14 - DNA, 3114 bp, Artificial sequence
  source 1..3114: mol_type = other DNA
taatacgactcactataggacatttgcttctgacacaactgtgttcactagcaacctcaaagagacaccgccaccatggtgagcaagggcgaggagctgttcaccggggtggtgcccatcctggtcgagctggacggcgacgtaaacggccacaagttcagcgtgtccggcgagggcgagggcgatgccacctacggcaagctgaccctgaagttcatctgcaccaccggcaagctgcccgtgccctggcccaccctcgtgaccaccctgacctacggcgtgcagtgcttcagccgctaccccgaccacatgaagcagcacgacttcttcaagtccgccatgcccgaaggctacgtccaggagcgcaccatcttcttcaaggacgacggcaactacaagacccgcgccgaggtgaagttcgagggcgacaccctggtgaaccgcatcgagctgaagggcatcgacttcaaggaggacggcaacatcctggggcacaagctggagtacaactacaacagccacaacgtctatatcatggccgacaagcagaagaacggcatcaaggtgaacttcaagatccgccacaacatcgaggacggcagcgtgcagctcgccgaccactaccagcagaacacccccatcggcgacggccccgtgctgctgcccgacaaccactacctgagcacccagtccgccctgagcaaagaccccaacgagaagcgcgatcacatggtcctgctggagttcgtgaccgccgccgggatcactctcggcatggacgagctgtacaagggaagcggagccacgaacttctctctgttaaagcaagcaggagatgttgaagaaaaccccgggcctatttatcctgctctggccgggggcggaggaggcggcggccaggtgggaagacagctggccattattggggatgccattaatagatgagctggagcctcggtagccgttcctcctgcccgctgggcctcccaacgggccctcctcccctccttgcaccggcccttcctggtctttgaataaagtctgagtgggcggaaaaaaaaaaaaaaaaaaaaaaaaaaaaaatgaagagccgtacgggcgcgcctaggcgcgattccgcttcctcgctcactgactcgctgcgctcggtcgttcggctgcggcgagcggtatcagctcactcaaaggcggtaatacggttatccacagaatcaggggataacgcaggaaagaacatgtgagcaaaaggccagcaaaaggccaggaaccgtaaaaaggccgcgttgctggcgtttttccataggctccgcccccctgacgagcatcacaaaaatcgacgctcaagtcagaggtggcgaaacccgacaggactataaagataccaggcgtttccccctggaagctccctcgtgcgctctcctgttccgaccctgccgcttaccggatacctgtccgcctttctcccttcgggaagcgtggcgctttctcatagctcacgctgtaggtatctcagttcggtgtaggtcgttcgctccaagctgggctgtgtgcacgaaccccccgttcagcccgaccgctgcgccttatccggtaactatcgtcttgagtccaacccggtaagacacgacttatcgccactggcagcagccactggtaacaggattagcagagcgaggtatgtaggcggtgctacagagttcttgaagtggtggcctaactacggctacactagaagaacagtatttggtatctgcgctctgctgaagccagttaccttcggaaaaagagttggtagctcttgatccggcaaacaaaccaccgctggtagcggtggtttttttgtttgcaagcagcagattacgcgcagaaaaaaaggatctcaagaagatcctttgatcttttctacggggtctgacgctcagtggaacgaaaactcacgttaagggattttggtcatgagattatcaaaaaggatcttcacctagatccttttaaattaaaaatgaagttttaaatcaatctaaagtatatatgagtaaacttggtctgacagttaccaatgcttaatcagtgaggcacctatctcagcgatctgtctatttcgttcatccatagttgcctgactccccgtcgtgtagataactacgatacgggagggcttaccatctggccccagtgctgcaatgataccgcgagatccacgctcaccggctccagatttatcagcaataaaccagccagccggaagggccgagcgcagaagtggtcctgcaactttatccgcctccatccagtctattaattgttgccgggaagctagagtaagtagttcgccagttaatagtttgcgcaacgttgttgccattgctacaggcatcgtggtgtcacgctcgtcgtttggtatggcttcattcagctccggttcccaacgatcaaggcgagttacatgatcccccatgttgtgcaaaaaagcggttagctccttcggtcctccgatcgttgtcagaagtaagttggccgcagtgttatcactcatggttatggcagcactgcataattctcttactgtcatgccatccgtaagatgcttttctgtgactggtgagtactcaaccaagtcattctgagaatagtgtatgcggcgaccgagttgctcttgcccggcgtcaatacgggataataccgcgccacatagcagaactttaaaagtgctcatcattggaaaacgttcttcggggcgaaaactctcaaggatcttaccgctgttgagatccagttcgatgtaacccactcgtgcacccaactgatcttcagcatcttttactttcaccagcgtttctgggtgagcaaaaacaggaaggcaaaatgccgcaaaaaagggaataagggcgacacggaaatgttgaatactcatactcttcctttttcaatattattgaagcatttatcagggttattgtctcatgagcggatacatatttgaatgtatttagaaaaataaacaaataggggttccgcgcacatttccccgaaaagtgccacctgacgtctaagaaaccattattatcatgacattaacctataaaaataggcgtatcacgaggccctttcgtc

SEQ ID NO: 15 - RNA, 1650 nt, Artificial sequence
  source 1..1650: mol_type = mRNA
atggaagacgccaaaaacataaagaaaggcccggcgccattctatcctctagaggatggaaccgctggagagcaactgcataaggctatgaagagatacgccctggttcctggaacaattgcttttacagatgcacatatcgaggtgaacatcacgtacgcggaatacttcgaaatgtccgttcggttggcagaagctatgaaacgatatgggctgaatacaaatcacagaatcgtcgtatgcagtgaaaactctcttcaattctttatgccggtgttgggcgcgttatttatcggagttgcagttgcgcccgcgaacgacatttataatgaacgtgaattgctcaacagtatgaacatttcgcagcctaccgtagtgtttgtttccaaaaaggggttgcaaaaaattttgaacgtgcaaaaaaaattaccaataatccagaaaattattatcatggattctaaaacggattaccagggatttcagtcgatgtacacgttcgtcacatctcatctacctcccggttttaatgaatacgattttgtaccagagtcctttgatcgtgacaaaacaattgcactgataatgaattcctctggatctactgggttacctaagggtgtggcccttccgcatagaactgcctgcgtcagattctcgcatgccagagatcctatttttggcaatcaaatcgttccggatactgcgattttaagtgttgtcccattccatcacggttttggaatgtttactacactcggatatttgatatgtggatttcgagtcgtcttaatgtatagatttgaagaagagctgtttttacgatcccttcaggattacaaaattcaaagtgcgttgctagtaccaaccctattttcattcttcgccaaaagcactctgattgacaaatacgatttatctaatttacacgaaattgcttctgggggcgcacctctttcgaaagaagtcggggaagcggttgcaaaacgcttccatcttccagggatacgacaaggatatgggctcactgagactacatcagctattctgattacacccgagggggatgataaaccgggcgcggtcggtaaagttgttccattttttgaagcgaaggttgtggatctggataccgggaaaacgctgggcgttaatcagagaggcgaattatgtgtcagaggacctatgattatgtccggttatgtaaacaatccggaagcgaccaacgccttgattgacaaggatggatggctacattctggagacatagcttactgggacgaagacgaacacttcttcatagttgaccgcttgaagtctttaattaaatacaaaggatatcaggtggcccccgctgaattggaatcgatattgttacaacaccccaacatcttcgacgcgggcgtggcaggtcttcccgacgatgacgccggtgaacttcccgccgccgttgttgttttggagcacggaaagacgatgacggaaaaagagatcgtggattacgtcgccagtcaagtaacaaccgcgaaaaagttgcgcggaggagttgtgtttgtggacgaagtaccgaaaggtcttaccggaaaactcgacgcaagaaaaatcagagagatcctcataaaggccaagaagggcggaaagtccaaattg